European Patent Specification EP 3 962 510 B1, published August 28, 2024. Title: NOVEL SELECTIVE ACKR3 MODULATORS AND USES THEREOF. Applicant: Luxembourg Institute of Health. The sequence listing filed with the application follows.

SEQUENCE LISTING (76 sequences)

SEQ ID NO: 1 - protein, 8 aa, Artificial Sequence
  consensus sequence 1
  SITE (4)..(4): Xaa is Phe or Trp
  SITE (8)..(8): Xaa is Lys, Val or Phe
FGGXMRRX

SEQ ID NO: 2 - protein, 9 aa, Artificial Sequence
  consensus sequence 2
  SITE (4)..(4): Xaa is Phe or Trp
  SITE (8)..(8): Xaa is Lys, Val or Phe
  SITE (9)..(9): Xaa can be any amino acid
FGGXMRRXX

SEQ ID NO: 3 - protein, 8 aa, Artificial Sequence
  peptide 1 - LIH383
FGGFMRRK

SEQ ID NO: 4 - protein, 9 aa, Artificial Sequence
  peptide 2
FGGFMRRKR

SEQ ID NO: 5 - protein, 9 aa, Artificial Sequence
  peptide 3
FGGFMRRVR

SEQ ID NO: 6 - protein, 8 aa, Artificial Sequence
  peptide 4
FGGWMRRK

SEQ ID NO: 7 - protein, 10 aa, Artificial Sequence
  consensus sequence 3
  SITE (4)..(4): Xaa is Phe or Trp
  SITE (8)..(8): Xaa is Lys, Val or Phe
  SITE (9)..(9): Xaa can be any amino acid
  SITE (10)..(10): Xaa can be any amino acid
FGGXMRRXXX

SEQ ID NO: 8 - protein, 11 aa, Artificial Sequence
  consensus sequence 4
  SITE (4)..(4): Xaa is Phe or Trp
  SITE (8)..(8): Xaa is Lys, Val or Phe
  SITE (9)..(9): Xaa can be any amino acid/
  SITE (10)..(10): Xaa can be any amino acid
  SITE (11)..(11): Xaa can be any amino acid
FGGXMRRXXXX

SEQ ID NO: 9 - protein, 12 aa, Artificial Sequence
  consensus sequence 5
  SITE (4)..(4): Xaa is Phe or Trp
  SITE (8)..(8): Xaa is Lys, Val or Phe
  SITE (9)..(9): Xaa can be any amino acid
  SITE (10)..(10): Xaa can be any amino acid
  SITE (11)..(11): Xaa can be any amino acid
  SITE (12)..(12): Xaa can be any amino acid
  SITE (12)..(12): Xaa can be any amino acid
FGGXMRRXXXXX

SEQ ID NO: 10 - protein, 9 aa, Artificial Sequence
  peptide 5
FGGWMRRVR

SEQ ID NO: 11 - protein, 9 aa, Artificial Sequence
  peptide 6
FGGWMRRKR

SEQ ID NO: 12 - protein, 5 aa, Artificial Sequence
  consensus sequence 6
  SITE (1)..(1): Xaa is Phe or Tyr
  SITE (5)..(5): Xaa is Leu or Met
XGGFX

SEQ ID NO: 13 - protein, 13 aa, Homo sapiens
  SITE (1)..(1): CH2-NH substituted
  SITE (13)..(13): NH2 substituted
FGGFTGARKSARK

SEQ ID NO: 14 - protein, 8 aa, Artificial Sequence [sequence omitted]

SEQ ID NO: 15 - protein, 5 aa, Artificial Sequence
  consensus sequence 7
  SITE (5)..(5): Xaa is Leu or Met
YGGFX

SEQ ID NO: 16 - protein, 5 aa, Artificial Sequence
  DADLE
  SITE (2)..(2): D-isomer of Ala
  SITE (5)..(5): D-isomer of Leu
YAGFL

SEQ ID NO: 17 - protein, 5 aa, Artificial Sequence
  DAMGO
  SITE (1)..(1): hydrogen substituted
  SITE (2)..(2): D-isomer of Ala
  SITE (4)..(4): N-methyl substituted
  SITE (5)..(5): OH-substituted
YAGFG

SEQ ID NO: 18 - protein, 17 aa, Homo sapiens
YGGFLRRIRPKLKWDNQ

SEQ ID NO: 19 - protein, 16 aa, Homo sapiens
GGFLRRIRPKLKWDNQ

SEQ ID NO: 20 - protein, 12 aa, Homo sapiens
  SITE (12)..(12): NH2-substituted
GGFLRRIRPKLK

SEQ ID NO: 21 - protein, 13 aa, Homo sapiens
YGGFLRRIRPKLK

SEQ ID NO: 22 - protein, 13 aa, Homo sapiens
YGGFLRRQFKVVT

SEQ ID NO: 23 - protein, 29 aa, Homo sapiens
YGGFLRRQFKVVTRSQEDPNAYSGELFDA

SEQ ID NO: 24 - protein, 32 aa, Homo sapiens
YGGFLRRIRPKLKWDNQKRYGGFLRRQFKVVT

SEQ ID NO: 25 - protein, 5 aa, Homo sapiens
YGGFM

SEQ ID NO: 26 - protein, 22 aa, Homo sapiens
YGGFMRRVGRPEWWMDYQKRYG

SEQ ID NO: 27 - protein, 17 aa, Homo sapiens
FGGFTGARKSARKLANQ

SEQ ID NO: 28 - protein, 13 aa, Homo sapiens
  SITE (13)..(13): NH2 substituted
FGGFTGARKSARK

SEQ ID NO: 29 - protein, 4 aa, Homo sapiens
  SITE (4)..(4): NH2 substituted
YPWF

SEQ ID NO: 30 - protein, 4 aa, Homo sapiens
  SITE (4)..(4): NH2 substituted
YPFF

SEQ ID NO: 31 - protein, 32 aa, Homo sapiens
YGGFMTSEKSQTPLVTLFKNAIIIKNAYKKGE

SEQ ID NO: 32 - protein, 8 aa, Artificial Sequence [sequence omitted]

SEQ ID NO: 33 - protein, 8 aa, Artificial Sequence
  peptide 8
KGGFMRRV

SEQ ID NO: 34 - protein, 8 aa, Artificial Sequence
  peptide 9
AGGFMRRV

SEQ ID NO: 35 - protein, 8 aa, Artificial Sequence
  peptide 10 - mother peptide
FGGFMRRV

SEQ ID NO: 36 - protein, 8 aa, Artificial Sequence
  peptide 11
NGGFMRRV

SEQ ID NO: 37 - protein, 8 aa, Artificial Sequence
  peptide 12
LGGFMRRV

SEQ ID NO: 38 - protein, 8 aa, Artificial Sequence
  peptide 13
YAGFMRRV

SEQ ID NO: 39 - protein, 8 aa, Artificial Sequence
  peptide 14
YSGFMRRV

SEQ ID NO: 40 - protein, 8 aa, Artificial Sequence
  peptide 15
YRGFMRRV

SEQ ID NO: 41 - protein, 8 aa, Artificial Sequence
  peptide 16
YGAFMRRV

SEQ ID NO: 42 - protein, 8 aa, Artificial Sequence
  peptide 17
YGSFMRRV

SEQ ID NO: 43 - protein, 8 aa, Artificial Sequence
  peptide 18
YGGYMRRV

SEQ ID NO: 44 - protein, 8 aa, Artificial Sequence
  peptide 19
YGGWMRRV

SEQ ID NO: 45 - protein, 8 aa, Artificial Sequence
  peptide 20
YGGLMRRV

SEQ ID NO: 46 - protein, 8 aa, Artificial Sequence
  peptide 21
YGGAMRRV

SEQ ID NO: 47 - protein, 8 aa, Artificial Sequence
  peptide 22
YGGFLRRV

SEQ ID NO: 48 - protein, 8 aa, Artificial Sequence
  peptide 23
YGGFARRV

SEQ ID NO: 49 - protein, 8 aa, Artificial Sequence
  peptide 24
YGGFKRRV

SEQ ID NO: 50 - protein, 8 aa, Artificial Sequence
  peptide 25
YGGFQRRV

SEQ ID NO: 51 - protein, 8 aa, Artificial Sequence
  peptide 26
YGGFFRRV

SEQ ID NO: 52 - protein, 8 aa, Artificial Sequence
  peptide 27
YGGFNRRV

SEQ ID NO: 53 - protein, 8 aa, Artificial Sequence
  peptide 28
YGGFMARV

SEQ ID NO: 54 - protein, 8 aa, Artificial Sequence
  peptide 29
YGGFMKRV

SEQ ID NO: 55 - protein, 8 aa, Artificial Sequence
  peptide 30
YGGFMRAV

SEQ ID NO: 56 - protein, 8 aa, Artificial Sequence
  peptide 31
YGGFMRKV

SEQ ID NO: 57 - protein, 8 aa, Artificial Sequence
  peptide 32
YGGFMRRL

SEQ ID NO: 58 - protein, 8 aa, Artificial Sequence
  peptide 33
YGGFMRRI

SEQ ID NO: 59 - protein, 8 aa, Artificial Sequence
  peptide 34
YGGFMRRA

SEQ ID NO: 60 - protein, 8 aa, Artificial Sequence
  peptide 35
YGGFMRRF

SEQ ID NO: 61 - protein, 8 aa, Artificial Sequence
  peptide 36
YGGFMRRK

SEQ ID NO: 62 - protein, 8 aa, Artificial Sequence
  peptide 37
YGGFMRRQ

SEQ ID NO: 63 - protein, 7 aa, Artificial Sequence
  peptide 38
GGFMRRV

SEQ ID NO: 64 - protein, 9 aa, Artificial Sequence
  peptide 39
AYGGFMRRV

SEQ ID NO: 65 - protein, 9 aa, Artificial Sequence
  peptide 40
YGGFMRRVA

SEQ ID NO: 66 - protein, 9 aa, Artificial Sequence
  peptide 41
YGGFMRRVR

SEQ ID NO: 67 - protein, 9 aa, Artificial Sequence
  peptide 42
YGGFMRRVC

SEQ ID NO: 68 - protein, 8 aa, Artificial Sequence
  peptide 43
FGGWMRRV

SEQ ID NO: 69 - protein, 8 aa, Artificial Sequence
  peptide 44
FGGFMRRF

SEQ ID NO: 70 - protein, 9 aa, Artificial Sequence
  peptide 45
FGGFMRRFR

SEQ ID NO: 71 - protein, 9 aa, Artificial Sequence
  peptide 46
FGGWMRRFR

SEQ ID NO: 72 - protein, 8 aa, Artificial Sequence
  peptide 47
FGGWMRRF

SEQ ID NO: 73 - protein, 4 aa, Homo sapiens
GRPE

SEQ ID NO: 74 - protein, 5 aa, Homo sapiens
GRPEW

SEQ ID NO: 75 - protein, 6 aa, Homo sapiens
GRPEWW

SEQ ID NO: 76 - protein, 7 aa, Homo sapiens
GRPEWWM